European Patent Application EP 4 455 286 A2, published October 30, 2024. Title: ENHANCING FORMATION OF HMOS BY MODIFYING LACTOSE IMPORT IN THE CELL. Applicant: DSM IP Assets B.V. Application EP PCT/EP2022/063311, filed May 17, 2022. The sequence listing filed with the application follows.

SEQUENCE LISTING (103 sequences)

SEQ ID NO: 1 - protein, 417 aa, Escherichia coli [sequence omitted]

SEQ ID NO: 2 - DNA, 1254 bp, Escherichia coli K-12
  misc_feature 1..1254: note = Nucleic acid sequence encoding LacY, GenBank ID: NC_000913.3
  source 1..1254: mol_type = other DNA
atgtactatttaaaaaacacaaacttttggatgttcggtttattctttttcttttacttttttatcatgggagcctacttcccgtttttcccgatttggctacatgacatcaaccatatcagcaaaagtgatacgggtattatttttgccgctatttctctgttctcgctattattccaaccgctgtttggtctgctttctgacaaactcgggctgcgcaaatacctgctgtggattattaccggcatgttagtgatgtttgcgccgttctttatttttatcttcgggccactgttacaatacaacattttagtaggatcgattgttggtggtatttatctaggcttttgttttaacgccggtgcgccagcagtagaggcatttattgagaaagtcagccgtcgcagtaatttcgaatttggtcgcgcgcggatgtttggctgtgttggctgggcgctgtgtgcctcgattgtcggcatcatgttcaccatcaataatcagtttgttttctggctgggctctggctgtgcactcatcctcgccgttttactctttttcgccaaaacggatgcgccctcttctgccacggttgccaatgcggtaggtgccaaccattcggcatttagccttaagctggcactggaactgttcagacagccaaaactgtggtttttgtcactgtatgttattggcgtttcctgcacctacgatgtttttgaccaacagtttgctaatttctttacttcgttctttgctaccggtgaacagggtacgcgggtatttggctacgtaacgacaatgggcgaattacttaacgcctcgattatgttctttgcgccactgatcattaatcgcatcggtgggaaaaacgccctgctgctggctggcactattatgtctgtacgtattattggctcatcgttcgccacctcagcgctggaagtggttattctgaaaacgctgcatatgtttgaagtaccgttcctgctggtgggctgctttaaatatattaccagccagtttgaagtgcgtttttcagcgacgatttatctggtctgtttctgcttctttaagcaactggcgatgatttttatgtctgtactggcgggcaatatgtatgaaagcatcggtttccagggcgcttatctggtgctgggtctggtggcgctgggcttcaccttaatttccgtgttcacgcttagcggccccggcccgctttccctgctgcgtcgtcaggtgaatgaagtcgcttaa

SEQ ID NO: 3 - protein, 433 aa, Escherichia coli
  REGION 1..433: note = Lactose permease, GenBank ID: WP_042094275.1
MYYLKNTNFWMFGLFFFFYFFIMGAYFPFFPIWLHDINHISKSDTGIIFAAISLFSLLFQPLFGLLSDKLGLRKYLLWIITGMLVMFAPFFIFIFGPLLQYNILVGSIVGGIYLGFCFNAGAPAVEAFIEKVSRRSNFEFGRARMFGCVGWALCASIVGIMFTINNQFVFWLGSGCALILAVLLFFAKTDAPSSATVANAVGANHSAFSLKLALELFRQPKLWFLSLYVIGVSCTYDVFDQQFANFFTSFFATGEQGTRVFGYVTTMGELLNASIMFFAPLIINRIGGKNALLLAGTIMSVRIIGSSFATSALEVVILKTLHMFEVPFLLVGCFKYITSQFEVRFSATIYLVCFCFFKQLAMIFMSVLAGNMYESIGFQGAYLVLGLVALGFTLISVFTLSGPGPLSLLRRQVNEVAYGCGASALSDQHIRAE

SEQ ID NO: 4 - protein, 417 aa, Proteobacteria [sequence omitted]

SEQ ID NO: 5 - protein, 417 aa, Campylobacter jejuni
  REGION 1..417: note = Lactose permease GenBank ID: WP_089607162.1
MYYLKNTNFWMFGLFFFFYFFIMGAYFPFFPIWLHDINHISKSDTGIIFAAISLFSLLFQPLFGLLSDKLGLRKYLLWIITGMLVMFAPFFIFIFGPLLQYNILVGSIVGGIYLGFCFNAGAPAVEAFIEKVSRRSNFEFGRARMFGCVGWALCASIVGIMFTINNQFVFWLGSGCCLILAVLLFFAKTDAPSSATVANAVGANHSAFSLKLALELFRQPKLWFLSLYVIGVSCTYDVFDQQFANFFTSFFATGEQGTRVFGYVTTMGELLNASIMFFAPLIINRIGGKNALLLAGTIMSVRIIGSSFATSALEVVILKTLHMFEVPFLLVGCFKYITSQFEVRFSATIYLVCFCFFKQLAMIFMSVLAGNMYESIGFQGAYLVLGLVALGFTLISVFTLSGPGPLSLLRRQVNEVA

SEQ ID NO: 6 - protein, 417 aa, Klebsiella pneumoniae
  REGION 1..417: note = Lactose permease, GenBank ID: WP_152280604.1
MYYLKNTNFWMFGLFFFFYFFIMGAYFPFFPIWLHDINHISKSDTGIIFAAISLFSLLFQPLFGLLSDKLGLRKYLLWIITGMLVMFAPFFIFIFGPLLQYNILVGSIVGGIYLGFCFNAGAPAVEAFIEKVSRRSNFEFGRARMFGCVGWALCASIVGIMFTINNQFVFWLGSGCALILAVLLFFAKTDAPSSATVANAVGANHSAFSLKLALELFRQPKLWFLSLYVIGVSCTYDVFDQQFANFFTSFFATGEQGTRVFGYVTTMGELLNASIMFFAPLIINRIGGKNALLLAGTIMSVRIIGSSFATSALEVVILKTLHMFEVPFLLVGCFKYITSQFEVRFSATIYLVCFCFFKQLAMIFMSILAGNMYESIGFQGAYLVLGLVALGFTLISVFTLSGPGPLSLLRRKVNEVA

SEQ ID NO: 7 - protein, 417 aa, Cronobacter sakazakii
  REGION 1..417: note = Lactose permease, GenBank ID: EGT4952364.1
MYYLKNTNFWMFGLFFFFYFFIMGAYFPFFPIWLHDINHISKSDTGIIFAAISLFSLLFQPLFGLLSDKLGLRKYLLWIITGMLVMFAPFFIFIFGPLLQYNILVGSIVGGIYLGFCFNAGAPAVEAFIEKVSRRSNFEYGRARMFGCVGWALCASIVGIMFTINNQFVFWLGSGCAFILAVLLFFAKTDAPSSATVANAVGANHSAFSLKLALELFRQPKLWFLSLYVIGVSCTYDVFDQQFANFFTSFFATGEQGTRVFGYVTTMGELLNASIMFFAPLIINRIGGKNALLLAGTIMSVRIIGSSFATSALEVVILKTLHMLEVPFLLVGCFKYITSQFEVRFSATIYLVCFCFFKQLAMIFMSILAGNMYESIGFQGAYLVLGLVALGFTLISVFTLSGPGPLSLLRRQVNEVA

SEQ ID NO: 8 - protein, 417 aa, Citrobacter freundii
  REGION 1..417: note = Lactose permease, GenBank ID NO: WP_134216118.1
MYYLKNTNFWMFGFFFFFYFFIMGAYFPFFPIWLHEVNHISKGDTGIIFACISLFSLLFQPIFGLLSDKLGLRKHLLWVITGMLVMFAPFFIYVFGPLLQVNILLGSIVGGIYLGFIYNAGAPAIEAYIEKASRRSNFEFGRARMFGCVGWALCASIAGIMFTINNQFVFWLGSGCAVILALLLLFSKTDAPSSAKVADAVGANNSAFSLKLALELFKQPKLWFLSLYVVGVSCTYDVFDQQFANFFTSLFATGEQGTRVFGYVTTMGELLNASIMFFAPLIVNRIGGKNALLLAGTIMSVRIIGSSFATTALEVVILKTLHMFEIPFLIVGCFKYITSQFEVRFSATIYLVCFCFFKQLAMIFMSVLAGKMYESIGFQGAYLVLGIIALSFTLISVFTLSGPGPFSLLRRRESVAL

SEQ ID NO: 9 - protein, 418 aa, Citrobacter freundii
  REGION 1..418: note = Lactose permease, GenBank ID: EDI1749185.1
MYYLKNTNFWMLGFFFFFYFFIMGAYFPFFPIWLHDINHISKGDTGIIFACISLFSLLFQPVFGLMSDKLGLRKNLLWIITGMLVMFAPFFIYVFGPLLHFNILLGSIVGGIYLGFIYNAGAPAIEAYIEKASRRSHFEFGRARMFGCVGWALCASIVGVMFTINNEFVFWLGSGCAVILALLLFFSRTDSGSSAVVADAVGANSSPFSLKLALELFKQPKLWFLSLYVVGVSCTYDVFDQQFANFFTSFFASGEQGTRVFGYVTTMGELLNACIMFFAPFIVNRIGGKNALLMAGIIMSVRIIGSSFATTAGEVVILKTLHMFEIPFLIVGCFKYITSQFEVRFSATIYLVCFCFFKQLAMIFMSVLAGNMYEKIGFQGAYLVLGLIALVFTLISVATLSGAGPLAVMRVSQQKSAS

SEQ ID NO: 10 - protein, 423 aa, Rouxiella badensis
  REGION 1..423: note = Lactose permease, GenBank ID: WP_084912833.1
MYYIKNTNFWTFGLFFFFYFFIMGAYFPFFPIWLHDINHINQSDTGIIFASISFFSLVFQPLFGLLSDKLGLKKHLLWIITGMLVMFAPFFIYVFGPLLKTNILLGSIVGGVYLGFIYNGGAPAIEAYIEKVSRRSSFEFGRARMFGCVGWAICASVVGIMFTINSQFVFWLGSGCAVILAVLLLVAKPAVGATAKVANELGANSKPFSLRLAAELLKDKKLWFLGLYVVGVSCTYEVFDQQFANFFTSFFSSADEGTRVFGYITTMGELLNALVMFFAPLIVNRIGGKNALLLAGIIMSVRIIGSSFASTPVEVVVLKTLHMFEVPFLIVGCFKYITSVFEVRFSATIYLVCFCFFKQIAMIFMSVFAGDMYGKIGFHGTYLILGLIALAFTLLSVFTLSGRGPLQAFKPVARTVEKPVSNV

SEQ ID NO: 11 - protein, 417 aa, Serratia marcescens
  REGION 1..417: note = Lactose permease, GenBank ID: WP_103826752.1
MYYLKNTNFWMFGLFFFFYFFFMGAYFPFFPIWLHDINHISKSDTGIIFAAISLFSLLFQPLFGLLSDKLGLRKYLLWIITGMLVMFAPFFIFIFGPLLQYNILVGSIVGGIYLGFCFNAGAPAVEAFIEKVSRRSNFEYGRARMFGCVGWALCASIVGIMFTINNQFVFWLGSGCAFILAVLLFFAKTDAPSSATVANAVGANHSAFSLKLALELFRQPKLWFLSLYVIGVSCTYDVFDQQFANFFTSFFATGEQGTRVFGYVTTMGELLNASIMFFAPLIINRIGGKNALLLAGTIMSVRIIGSSFATSALEVVILKTLHMFEVPFLLVGCFKYITSQFEVRFSATIYLVCFCFFKQLAMIFMSILAGNMYESIGFQGAYLVLGLVALGFTLISVFTLSGPGPLSLLRRQVNEVA

SEQ ID NO: 12 - protein, 420 aa, Serratia fonticola
  REGION 1..420: note = Lactose permease, GenBank ID: WP_021804673.1
MYYLKNTNFWMFGLFFFFYFFIMGAYFPFFPIWLHDINQVSKSDTGIIFASISFFSLLFQPIFGLLSDKLGLRKHLLWIITGMLILFAPFFIYVFGPLLRTNIVLGSIAGGIYLGFIYNGGAPAIEAYIEKVSRRSSFEFGRARLFGCVGWALCASVVGIMFTINNEFVFWLGSGCAVILAILLLIAKPEAGSTAQVADKLGANSKPFNLRLAFELLKDSKLWFLALYVVGVSCTYDVFDQQFANFFTSFFSSSEQGTRVFGYVTTMGELLNASIMFFAPLIVNRIGGKNALLLAGLIMSIRIIGSSFASTPVEVVILKTLHMFEIPFLIVGCFKYITSVFEVRFSATIYLVCFCFFKQLAIMFMSVFAGNMYEKVGFHGTYLILGLIALSFTLISVFTLSGRGPLSAFKPEPEAVRNMA

SEQ ID NO: 13 - protein, 423 aa, Rouxiella silvae
  REGION 1..423: note = Lactose permease, GenBank ID: WP_084984472.1
MNYMRNTNFWTFGLFFFFYFFIMGAYFPFFPIWLHDINHINQSDTGIIFACISFFSLVFQPLFGLLSDKLGLKKHLLWIITGMLVLFAPFFIYVFGPLLQTNILLGSIVGGIYLGFIYNGGAPAIEAYIEKVSRRSSFEFGRARMFGCVGWAICASVVGIMFTINNQFVFWLGSGCAVILAILLLIAKPAVGASAKVANELGANSKPFNLRLAAELLKDKKLWFLGLYVVGVSCTYEVFDQQFANFFTSFFSSADQGTRVFGYITTLGELLNAFIMFFAPAIVNRIGGKNALLLAGAIMSVRIIGSSFASTPVEVVLLKTLHMFEIPFLIVGCFKYITSVFEVRFSATIYLVCFCFFKQIAMIFMSIFAGEMYGKVGFHGTYLILGLIALAFTLVSIFTLTGRGPLQAFKPSQRVSETRPVSP

SEQ ID NO: 14 - protein, 412 aa, Aeromonas
  REGION 1..412: note = Lactose permease, GenBank ID: WP_199428647.1
MFGAIFFLYFFIMGAYFPFFPIWLHDVNGISKAETGIVFGTISLFALLFQPVFGLVSDKLGLKKHLLWIIIGLLVFFAPFFLYVLAPLLKLNIYLGSIVGGMYIGFVFAGGAPAIEAYVEKVSRSSQFEFGRARMFGAIGWALCASIVGIMFTINNEFVFWMGSAFAVVMAVLFYFINPGRGSTSEVLDSIGANQKGFSIKLAMRLLKQAKFWFFTLYVIGVACTYDVFDQQFANFFTAFFDTKEEGTRYFGYVTTMGELLNASIMFFAPLIVNRIGGKNALLIAGTIMSIRIIGSSFAETVSHVILLKTLHMLEVPFLLVGTFKYITSEFDVRFSATIWLIGYQFFKQLATMFMSVWAGSMYEVMGFRETYLVLGIIAATFTFISIFTLSGMGPLGLLKGRTMVSKKTASY

SEQ ID NO: 15 - protein, 425 aa, Yersinia pestis
  REGION 1..425: note = Lactose permease, GenBank ID: WP_046596210.1
MKISKTGNYTILFTVSFFIMASYYPFFPIWLHDINNLSKTDTGIVFGSISLFALAFQPIMGPLSDKLGLRKTLMWIIVGLLVLFAPFFIYVFSPLLKYNIFIGAIVGGCYLGFVFTGGSHAIEAYIEKVSRHSNFEYGRVRMFGCIGWALCATVVGILYTVNNQLIFWMASGCALILAVLLFFARPDRQSTAFVVDTLGANKAVFNLKNALALLRKRELWFFVMYIVGVACIYDVFDQQFANFFTSFFATKQQGTEIFGFVTTGGEILNATVMFFAPVIIARIGSKNALLLAGTIMSVRILGSAFATTATQVVFLKMLHMFEVPFLLVGSFKYITQVFEVRFSATVYLIGFCFSKQLSMMFMSVFAGRMYGSMGYQDTYMVLGVIVLSFTLISAFTLSGRSAVANLASRLKEDPSVTPPVSQPQS

SEQ ID NO: 16 - protein, 587 aa, Kluyveromyces lactis
  REGION 1..587: note = Lactose permease, GenBank ID: XP_452193.1
MADHSSSSSSLQKKPINTIEHKDTLGNDRDHKEALNSDNDNTSGLKINGVPIEDAREEVLLPGYLSKQYYKLYGLCFITYLCATMQGYDGALMGSIYTEDAYLKYYHLDINSSSGTGLVFSIFNVGQICGAFFVPLMDWKGRKPAILIGCLGVVIGAIISSLTTTKSALIGGRWFVAFFATIANAAAPTYCAEVAPAHLRGKVAGLYNTLWSVGSIVAAFSTYGTNKNFPNSSKAFKIPLYLQMMFPGLVCIFGWLIPESPRWLVGVGREEEAREFIIKYHLNGDRTHPLLDMEMAEIIESFHGTDLSNPLEMLDVRSLFRTRSDRYRAMLVILMAWFGQFSGNNVCSYYLPTMLRNVGMKSVSLNVLMNGVYSIVTWISSICGAFFIDKIGRREGFLGSISGAALALTGLSICTARYEKTKKKSASNGALVFIYLFGGIFSFAFTPMQSMYSTEVSTNLTRSKAQLLNFVVSGVAQFVNQFATPKAMKNIKYWFYVFYVFFDIFEFIVIYFFFVETKGRSLEELEVVFEAPNPRKASVDQAFLAQVRATLVQRNDVRVANAQNLKEQEPLKSDADHVEKLSEAESV

SEQ ID NO: 17 - protein, 262 aa, Chromobacterium violaceum
  REGION 1..262: note = cvb3galT, -1,3-galactosyltransferase, GeneBank ID: WP_080969100.1
MDTIMIKRPLVSVILPVNKNNPHLEEAIQSIKNQTYKELELIIIANNCEDNFYSLLLKYQDQKTKIIRTSIKYLPFSLNLGVHLSQGEYIARMDSDDISVLDRIEKQVKRFLNTPELSILGSNVEYINEASESIGYSNYPLDHSSIVNSFPFRCNLAHPTIMVKKEVITTLGGYMYGSLSEDYDLWIRASRHGNFKFSNIDEPLLKYRIHKGQATNKSNAYNIFAFDSSLKIREFLLNGNVQYLLGAARGFFAFLYVRFIKK

SEQ ID NO: 18 - protein, 439 aa, synthetic construct
  REGION 1..439: note = galTK, -1,3-galactosyltransferase, homologous to GeneBank ID: BD182026.1
MISVYIISLKESQRRLDTEKLVLESNEKFKGRCVFQIFDAISPKHEDFEKFVQELYDSSSLLKSDWFHSDYCYQELLPQEFGCYLSHYLLWKECVKLNQPVVILEDDVALESNFMQALEDCLKSPFDFVRLYGHYWGGHKTNLCALPVYTETEEAEASIEKTPIENYEVTSPPPPNPTRDTQQDFITETQQDPKELSEPCKIAPQKISFNQVVFKKIKRKLNRFIGSILARTEVYKNIVAKYDDLTTKYDDLTTKYDDLTTKYDDLTTKYDDLNKNIAEKYDELMGKYESLLAKEVNIKETFWESRADSEKEALFLDHFYLTSVYVATTAGYYLTPKGAKTFIEATERFKIIEPVDMFINNPTYHDIANFTYVPCPVSLNKHAFNSTIQNAKKPDISLKPPKKSYFDNLFYHKFNARKCLKAFNKYSKQYAPLKTPKEV

SEQ ID NO: 19 - protein, 273 aa, Helicobacter pylori
  REGION 1..273: note = -1,4-gal-transferase, GalT, GenBank ID: WP_001262061.1
MRVFAISLNQKVCDTFGLVFRDTTTLLNSINATHHQAQIFDAIYSKTFEGGLHPLVKKHLHPYFITQNIKDMGITTNLISEVSKFYYALKYHAKFMSLGELGCYASHYSLWEKCIELNEAICILEDDITLKEDFKEGLDFLEKHIQELGYIRLMHLLYDASVKSEPLSHKNHEIQERVGIIKAYSEGVGTQGYVITPKIAKVFLKCSRKWVVPVDTIMDATFIHGVKNLVLQPFVIADDEQISTIARKEEPYSPKIALMRELHFKYLKYWQFV

SEQ ID NO: 20 - protein, 332 aa, Neisseria meningitidis
  REGION 1..332: note = lgtA, -1,3-N-acetyl-glucosaminyltransferase, GeneBank ID: WP_033911473.1
MQPLVSVLICAYNVEKYFAQSLAAVVNQTWRNLEILIVDDGSTDGTLAIAKDFQKRDSRIKILAQAQNSGLIPSLNIGLDELAKSGMGEYIARTDADDIAAPDWIEKIVGEMEKDRSIIAMGAWLEVLSEEKDGNRLARHHRHGKIWKKPTRPEDIADFFPFGNPIHNNTMIMRRSVIDGGLRYNTERDWAEDYQFWYDVSKLGRLAYYPEALVKYRLHANQVSSKYSIRQHEIAQGIQKTARNDFLQSMGFKTRFDSLEYRQIKAVAYELLEKHLPEEDFERARRFLYQCFKRTDTLPAGAWLDFAADGRMRRLFTLRQYFGILHRLLKNR

SEQ ID NO: 21 - protein, 334 aa, Pasteurella multocida
  REGION 1..334: note = pmnagT, -1,3-N-acetylglucosaminyl-transferase, GeneBankID: WP_014390683.1
MENKPLVSVLICAYNVEKYIEECINAVINQTYKNLEIIIVNDGSSDNTYFLLKKLAEKDNRIKILNFNNHIGIISALNEGLKEIAGEYIARTDSDDITKPDWIEKILTCMQNDPKIIAMGSYLTVLSEENNGSVLANHHKNKVEWKNPLEHKDIVEKMLFGNPIHNNSMVMRSEIYTKYHLIYDPDYHYAEDYKFWLEVSRIGKLANYPESLVYYRLHRNQTSSIHNSQQEINGKKLRLQALNYYLKDLGIDYQLPEKFLFKDIALLQEIFYERGMFRENIIRRIIYECYLSLGEYNYKDIYYFLINKNNFLSIKDKFKIIKKYLRPDKYSSTY

SEQ ID NO: 22 - protein, 330 aa, Haemophilus ducreyi
  REGION 1..330: note = HD0466, glycosyltransferase family 2 protein, GeneBank ID: WP_010944479.1
MTTLVSVLICAYNVEKYIDECLNAVIAQTYKNLEIIVVNDGSTDGTLAKLRQFEAKDPRVKIIDNIVNQGTSKSLNIGIQYCQGEIIARTDSDDIVDIHWIETLMRELDNSPETIAISAYLEFLAEKGNGSKLSRSRKHGKNAENPISSEAISQRMLFGNPVHNNVALVRRKVFSEYGLRFDPDYIHAEDYKFWFEVSKLGKMRTYPKALVKYRLHATQVSSAYNQKQRSIAKKIKREAISHYLQQYGIQLPEKLTIHDLFSIFSPQIELSLTVANKQELFWSLATSLSEYHFRDLLKIYSLDIFHQLSFKYKKRIFRKFLLPNRYPSVI

SEQ ID NO: 23 - protein, 302 aa, synthetic construct
  REGION 1..302: note = FutC ( -1,2-fucosyl-transferase)
MAFKVVQICGGLGNQMFQYAFAKSLQKHSNTPVLLDITSFDWSDRKMQLELFPIDLPYASAKEIAIAKMQHLPKLVRDALKCMGFDRVSQEIVFEYEPKLLKPSRLTYFFGYFQDPRYFDAISPLIKQTFTLPPPPENNKNNNKKEEEYQCKLSLILAAKNSVFVHIRRGDYVGIGCQLGIDYQKKALEYMAKRVPNMELFVFCEDLEFTQNLDLGYPFMDMTTRDKEEEAYWDMLLMQSCQHGIIANSTYSWWAAYLIENPEKIIIGPKHWLFGHENILCKEWVKIESHFEVKSQKYNALG

SEQ ID NO: 24 - protein, 292 aa, Sulfuriflexus mobilis
  REGION 1..292: note = Smob, -1,2-fucosyltransferase, GeneBank ID: WP_126455392.1
MIISQIIGGLGNQMFQYAAGRALSLVRGQPLLLDVTGFAGYGLHQGFELQRVFDCPIGIATEEDVRGILGWQFSAGIRRIVARPGMAAFRRKGFIVEPHFHYWPEIKNVPRDCYLLGYWQSERYFRAATADIRADFSFKSPLVNRNAETAAQIDQVNAISLHMRRGDYVNNPKTSATHGLCSLDYYQAAIKFVSERVEEPFFFIFSDDIAWVKANLKLDFPCQYVDHNHGAESFNDMHLMSLCQHHIIANSSFSWWGAWLNSDPKKIVLAPKKWFANKNNIKDLFPPGWVSL

SEQ ID NO: 25 - protein, 292 aa, Methylobacter tundripaludum
  REGION 1..292: note = Mtun, -1,2-fucosyltransferase, GeneBank ID: WP_031437198.1
MVITHLIGGLGNQMFQYAAGRAVSLERGVSLSLDISGFANYGLHQGFELQRIFNCTAEIANEADVRGILGWQSSPRIRQLLSRQNMAIFRREGFVVEPHFHYWQGIKSVPRDCYLTGYWQSEQYFLEAAAQIRADFTFKLPLDNQNIELAKQINAVNAVSLHVRRGDYANTPETTATHGLCSLDYYRVAIRHIAEQVQQPHFFVFSDDIAWVKNNLSIDFPCQYVDHNQGAESYNDMRLMSMCRHHIIANSSFSWWGAWLNPNVNKIVVAPSRWFAKQTDVRDLLPQGWIKQ

SEQ ID NO: 26 - protein, 425 aa, Helicobacter pylori
  REGION 1..425: note = FutA, -1,3-fucosyl-transferase, GenBank ID: NP_207177.1
MFQPLLDAFIESASIEKMASKSPPPPLKIAVANWWGDEEIKEFKKSVLYFILSQRYAITLHQNPNEFSDLVFSNPLGAARKILSYQNTKRVFYTGENESPNFNLFDYAIGFDELDFNDRYLRMPLYYAHLHYKAELVNDTTAPYKLKDNSLYALKKPSHHFKENHPNLCAVVNDESDLLKRGFASFVASNANAPMRNAFYDALNSIEPVTGGGSVRNTLGYKVGNKSEFLSQYKFNLCFENSQGYGYVTEKILDAYFSHTIPIYWGSPSVAKDFNPKSFVNVHDFNNFDEAIDYIKYLHTHPNAYLDMLYENPLNTLDGKAYFYQDLSFKKILDFFKTILENDTIYHKFSTSFMWEYDLHKPLVSIDDLRVNYDDLRVNYDRLLQNASPLLELSQNTTFKIYRKAYQKSLPLLRAVRKLVKKLGL

SEQ ID NO: 27 - protein, 478 aa, Helicobacter pylori NCTC 11639
  REGION 1..478: note = FucT, alpha1,3-fucosyltransferase, GenBank ID NO: AAB81031.1
MFQPLLDAYVESASIEKMASKSPPPLKIAVANWWGDEEIKEFKNSVLYFILSQRYTITLHQNPNEFSDLVFGNPLGSARKILSYQNAKRVFYTGENESPNFNLFDYAIGFDELDFNDRYLRMPLYYDRLHHKAESVNDTTAPYKLKDNSLYALKKPSHCFKEKHPNLCAVVNDESDPLKRGFASFVASNPNAPIRNAFYDALNSIEPVTGGGSVRNTLGYNVKNKNEFLSQYKFNLCFENTQGYGYVTEKIIDAYFSHTIPIYWGSPSVAKDFNPKSFVNVHDFKNFDEAIDYIKYLHTHKNAYLDMLYENPLNTLDGKAYFYQNLSFKKILAFFKTILENDTIYHDNPFIFCRDLNEPLVTIDDLRVNYDDLRVNYDDLRINYDDLRVNYDDLRINYDDLRVNYDDLRVNYDDLRINYDDLRVNYDDLRVNYERLLSKATPLLELSQNTTSKIYRKAYQKSLPLLRAIRRWVKKLGL

SEQ ID NO: 28 - protein, 432 aa, Helicobacter pylori
  REGION 1..432: note = FucTIII, alpha-1,4 fucosyltransferase, GenBank ID: AAR88243.1
MFQPLLDAYIDSTRLDETDYKPPLKIAVANWWGGVEEFKKSTLYFILSQRYTITLHRNPDKPADIVFGNPLGSARKILSYQNAKRVFYTGENEVPNFNLFDYAIGFDELDFNDRYLRMPLYYAHLHYEAELVNDTTSPYKIKDNSLYALKKPSHHFKENHPNLCAVVNNESDPLKRGFASFVASNPNAPKRNAFYDALNSIEPVTGGGSVKNTLGYNVKNKNEFLSQYKFNLCFENSQGYGYVTEKILDAYFSHTIPIYWGSPSVAKDFNPKSFVNVHDFNNFDEAIDHVRYLHTHPNAYLDMLYENPLNTLDGKAYFYQNLSFKKILDFFKTILENDTIYHCDAHNYSALHRDLNEPLVSIDDLRINYDDLRINYDDLRINYDDLRINYERLLQNASPLLELSQNTSFKIYRKAYQKSLPLLRAIRRWVKK

SEQ ID NO: 29 - protein, 483 aa, synthetic construct
  REGION 1..483: note = Pd2 ( -1,3-sialyl-transferase)
MCNSDNTSLKETVSSNSADVVETETYQLTPIDAPSSFLSHSWEQTCGTPILNESDKQAISFDFVAPELKQDEKYCFTFKGITGDHRYITNTTLTVVAPTLEVYIDHASLPSLQQLIHIIQAKDEYPSNQRFVSWKRVTVDADNANKLNIHTYPLKGNNTSPEMVAAIDEYAQSKNRLNIEFYTNTAHVFNNLPPIIQPLYNNEKVKISHISLYDDGSSEYVSLYQWKDTPNKIETLEGEVSLLANYLAGTSPDAPKGMGNRYNWHKLYDTDYYFLREDYLDVEANLHDLRDYLGSSAKQMPWDEFAKLSDSQQTLFLDIVGFDKEQLQQQYSQSPLPNFIFTGTTTWAGGETKEYYAQQQVNVINNAINETSPYYLGKDYDLFFKGHPAGGVINDIILGSFPDMINIPAKISFEVLMMTDMLPDTVAGIASSLYFTIPADKVNFIVFTSSDTITDREEALKSPLVQVMLTLGIVKEKDVLFWA

SEQ ID NO: 30 - protein, 342 aa, synthetic construct
  REGION 1..342: note = Nst ( -1,3-sialyl-transferase)
MERNAVSLLKEKLFNEEGEPVNLIFCYTILQMKVAERIMAQHPGERFYVVLMSENRNEKYDYYFNQIKDKAERAYFFHLPYGLNKSFNFIPTMAELKVKSMLLPKVKRIYLASLEKVSIAAFLSTYPDAEIKTFDDGTGNLIQSSSYLGDEFSVNGTIKRNFARMMIGDWSIAKTRNASDEHYTIFKGLKNIMDDGRRKMTYLPLFDASELKTGDETGGTVRILLGSPDKEMKEISEKAAKNFKIQYVAPHPRQTYGLSGVTTLNSPYVIEDYILREIKKNPHTRYEIYTFFSGAALTMKDFPNVHVYALKPASLPEDYWLKPVYALFTQSGIPILTFDDKN

SEQ ID NO: 31 - protein, 373 aa, Escherichia coli K-12 [sequence omitted]

SEQ ID NO: 32 - protein, 373 aa, Enterobacteriaceae [sequence omitted]

SEQ ID NO: 33 - protein, 321 aa, Escherichia coli K-12
  REGION 1..321: note = WcaG, GDP-L-fucose synthase
MSKQRVFIAGHRGMVGSAIRRQLEQRGDVELVLRTRDELNLLDSRAVHDFFASERIDQVYLAAAKVGGIVANNTYPADFIYQNMMIESNIIHAAHQNDVNKLLFLGSSCIYPKLAKQPMAESELLQGTLEPTNEPYAIAKIAGIKLCESYNRQYGRDYRSVMPTNLYGPHDNFHPSNSHVIPALLRRFHEATAQNAPDVVVWGSGTPMREFLHVDDMAAASIHVMELAHEVWLENTQPMLSHINVGTGVDCTIRELAQTIAKVVGYKGRVVFDASKPDGTPRKLLDVTRLHQLGWYHEISLEAGLASTYQWFLENQDRFRG

SEQ ID NO: 34 - protein, 321 aa, Enterobacteriaceae; identical to SEQ ID NO: 33
  REGION 1..321: note = WcaG, GDP-L-fucose synthase, GenBank ID: WP_000043654.1

SEQ ID NO: 35 - protein, 159 aa, Escherichia coli
  REGION 1..159: note = WcaH, GDP-mannose mannosyl hydrolase, GenBank ID: NP_416555.2
MFLRQEDFATVVRSTPLVSLDFIVENSRGEFLLGKRTNRPAQGYWFVPGGRVQKDETLEAAFERLTMAELGLRLPITAGQFYGVWQHFYDDNFSGTDFTTHYVVLGFRFRVSEEELLLPDEQHDDYRWLTSDALLASDNVHANSRAYFLAEKRTGVPGL

SEQ ID NO: 36 - protein, 159 aa, Escherichia; identical to SEQ ID NO: 35
  REGION 1..159: note = WcaH, GDP-mannose mannosyl hydrolase, GenBank ID: WP_001393539.1

SEQ ID NO: 37 - protein, 407 aa, Escherichia coli
  REGION 1..407: note = WcaI, colanic acid biosynthesis fucosyltransferase, GenBank ID: NP_416554.1
MKILVYGINYSPELTGIGKYTGEMVEWLAAQGHEVRVITAPPYYPQWQVGENYSAWRYKREEGAATVWRCPLYVPKQPSTLKRLLHLGSFAVSSFFPLMAQRRWKPDRIIGVVPTLFCAPGMRLLAKLSGARTVLHIQDYEVDAMLGLGLAGKGKGGKVAQLATAFERSGLHNVDNVSTISRSMMNKAIEKGVAAENVIFFPNWSEIARFQHVADADVDALRNQLDLPDNKKIILYSGNIGEKQGLENVIEAADRLRDEPLIFAIVGQGGGKARLEKMAQQRGLRNMQFFPLQSYDALPALLKMGDCHLVVQKRGAADAVLPSKLTNILAVGGNAVITAEAYTELGQLCETFPGIAVCVEPESVEALVAGIRQALLLPKHNTVAREYAERTLDKENVLRQFINDIRG

SEQ ID NO: 38 - protein, 407 aa, Escherichia; identical to SEQ ID NO: 37
  REGION 1..407: note = WcaI, colanic acid biosynthesis fucosyltransferase , GenBank ID: WP_000699693.1

SEQ ID NO: 39 - protein, 478 aa, Escherichia coli K-12
  REGION 1..478: note = ManC, mannose-1-phosphate guanylyltransferase, GenBank ID: NP_416553.1
MAQSKLYPVVMAGGSGSRLWPLSRVLYPKQFLCLKGDLTMLQTTICRLNGVECESPVVICNEQHRFIVAEQLRQLNKLTENIILEPAGRNTAPAIALAALAAKRHSPESDPLMLVLAADHVIADEDAFRAAVRNAMPYAEAGKLVTFGIVPDLPETGYGYIRRGEVSAGEQDMVAFEVAQFVEKPNLETAQAYVASGEYYWNSGMFLFRAGRYLEELKKYRPDILDACEKAMSAVDPDLNFIRVDEEAFLACPEESVDYAVMERTADAVVVPMDAGWSDVGSWSSLWEISAHTAEGNVCHGDVINHKTENSYVYAESGLVTTVGVKDLVVVQTKDAVLIADRNAVQDVKKVVEQIKADGRHEHRVHREVYRPWGKYDSIDAGDRYQVKRITVKPGEGLSVQMHHHRAEHWVVVAGTAKVTIDGDIKLLGENESIYIPLGATHCLENPGKIPLDLIEVRSGSYLEEDDVVRFADRYGRV

SEQ ID NO: 40 - protein, 478 aa, Escherichia; identical to SEQ ID NO: 39
  REGION 1..478: note = ManC, mannose-1-phosphate guanyltransferase, GenBank ID: WP_000079274.1

SEQ ID NO: 41 - protein, 456 aa, Escherichia coli K-12
  REGION 1..456: note = ManB, phosphomannomutase, GenBank ID: NP_416552.1
MKKLTCFKAYDIRGKLGEELNEDIAWRIGRAYGEFLKPKTIVLGGDVRLTSETLKLALAKGLQDAGVDVLDIGMSGTEEIYFATFHLGVDGGIEVTASHNPMDYNGMKLVREGARPISGDTGLRDVQRLAEANDFPPVDETKRGRYQQINLRDAYVDHLFGYINVKNLTPLKLVINSGNGAAGPVVDAIEARFKALGAPVELIKVHNTPDGNFPNGIPNPLLPECRDDTRNAVIKHGADMGIAFDGDFDRCFLFDEKGQFIEGYYIVGLLAEAFLEKNPGAKIIHDPRLSWNTVDVVTAAGGTPVMSKTGHAFIKERMRKEDAIYGGEMSAHHYFRDFAYCDSGMIPWLLVAELVCLKDKTLGELVRDRMAAFPASGEINSKLAQPVEAINRVEQHFSREALAVDRTDGISMTFADWRFNLRTSNTEPVVRLNVESRGDVPLMEARTRTLLTLLNE

SEQ ID NO: 42 - protein, 456 aa, Escherichia; identical to SEQ ID NO: 41
  REGION 1..456: note = ManB, phosphomannomutase, GenBank ID: WP_001350528.1

SEQ ID NO: 43 - protein, 546 aa, Escherichia coli K-12
  REGION 1..546: note = pgm, Phosphoglucomutase, GenBank ID: NP_415214.1
MAIHNRAGQPAQQSDLINVAQLTAQYYVLKPEAGNAEHAVKFGTSGHRGSAARHSFNEPHILAIAQAIAEERAKNGITGPCYVGKDTHALSEPAFISVLEVLAANGVDVIVQENNGFTPTPAVSNAILVHNKKGGPLADGIVITPSHNPPEDGGIKYNPPNGGPADTNVTKVVEDRANALLADGLKGVKRISLDEAMASGHVKEQDLVQPFVEGLADIVDMAAIQKAGLTLGVDPLGGSGIEYWKRIGEYYNLNLTIVNDQVDQTFRFMHLDKDGAIRMDCSSECAMAGLLALRDKFDLAFANDPDYDRHGIVTPAGLMNPNHYLAVAINYLFQHRPQWGKDVAVGKTLVSSAMIDRVVNDLGRKLVEVPVGFKWFVDGLFDGSFGFGGEESAGASFLRFDGTPWSTDKDGIIMCLLAAEITAVTGKNPQEHYNELAKRFGAPSYNRLQAAATSAQKAALSKLSPEMVSASTLAGDPITARLTAAPGNGASIGGLKVMTDNGWFAARPSGTEDAYKIYCESFLGEEHRKQIEKEAVEIVSEVLKNA

SEQ ID NO: 44 - protein, 553 aa, Escherichia coli
  REGION 1..553: note = pgm, phosphoglucomutase, GenBank ID: WP_001396326.1
MQTKDKAMAIHNRAGQPAQQSDLINVAQLTAQYYVLKPEAGNAEHAVKFGTSGHRGSAARHSFNEPHILAIAQAIAEERAKNGITGPCYVGKDTHALSEPAFISVLEVLAANGVDVIVQENNGFTPTPAVSNAILVHNKKGGPLADGIVITPSHNPPEDGGIKYNPPNGGPADTNVTKVVEDRANALLADGLKGVKRISLDEAMASGHVKEQDLVQPFVEGLADIVDMAAIQKAGLTLGVDPLGGSGIEYWKRIGEYYNLNLTIVNDQVDQTFRFMHLDKDGAIRMDCSSECAMAGLLALRDKFDLAFANDPDYDRHGIVTPAGLMNPNHYLAVAINYLFQHRPQWGKDVAVGKTLVSSAMIDRVVNDLGRKLVEVPVGFKWFVDGLFDGSFGFGGEESAGASFLRFDGTPWSTDKDGIIMCLLAAEITAVTGKNPQEHYNELAKRFGAPSYNRLQAAATSAQKAALSKLSPEMVSASTLAGDPITARLTAAPGNGASIGGLKVMTDNGWFAARPSGTEDAYKIYCESFLGEEHRKQIEKEAVEIVSEVLKNA

SEQ ID NO: 45 - protein, 302 aa, Escherichia coli K-12
  REGION 1..302: note = GalU, UTP-glucose-1-phosphate uridylyltransferase, GenBank: NP_415752.1
MAAINTKVKKAVIPVAGLGTRMLPATKAIPKEMLPLVDKPLIQYVVNECIAAGITEIVLVTHSSKNSIENHFDTSFELEAMLEKRVKRQLLDEVQSICPPHVTIMQVRQGLAKGLGHAVLCAHPVVGDEPVAVILPDVILDEYESDLSQDNLAEMIRRFDETGHSQIMVEPVADVTAYGVVDCKGVELAPGESVPMVGVVEKPKADVAPSNLAIVGRYVLSADIWPLLAKTPPGAGDEIQLTDAIDMLIEKETVEAYHMKGKSHDCGNKLGYMQAFVEYGIRHNTLGTEFKAWLEEEMGIKK

SEQ ID NO: 46 - protein, 302 aa, Enterobacteriaceae; identical to SEQ ID NO: 45
  REGION 1..302: note = GalU, UTP-glucose-1-phosphate uridylyltransferase, WP_000718995.1

SEQ ID NO: 47 - protein, 338 aa, Escherichia coli K-12
  REGION 1..338: note = GalE, UDP-glucose 4-epimerase, GenBank ID: NP_415280.3
MRVLVTGGSGYIGSHTCVQLLQNGHDVIILDNLCNSKRSVLPVIERLGGKHPTFVEGDIRNEALMTEILHDHAIDTVIHFAGLKAVGESVQKPLEYYDNNVNGTLRLISAMRAANVKNFIFSSSATVYGDQPKIPYVESFPTGTPQSPYGKSKLMVEQILTDLQKAQPDWSIALLRYFNPVGAHPSGDMGEDPQGIPNNLMPYIAQVAVGRRDSLAIFGNDYPTEDGTGVRDYIHVMDLADGHVVAMEKLANKPGVHIYNLGAGVGNSVLDVVNAFSKACGKPVNYHFAPRREGDLPAYWADASKADRELNWRVTRTLDEMAQDTWHWQSRHPQGYPD

SEQ ID NO: 48 - protein, 338 aa, Enterobacteriaceae; identical to SEQ ID NO: 47
  REGION 1..338: note = GalE, UDP-glucose 4-epimerase, GenBank ID: WP_001265438.1

SEQ ID NO: 49 - protein, 445 aa, Escherichia coli K-12
  REGION 1..445: note = GlmM, Phosphoglucosamine mutase, GenBank ID: NP_417643.1
MSNRKYFGTDGIRGRVGDAPITPDFVLKLGWAAGKVLARHGSRKIIIGKDTRISGYMLESALEAGLAAAGLSALFTGPMPTPAVAYLTRTFRAEAGIVISASHNPFYDNGIKFFSIDGTKLPDAVEEAIEAEMEKEISCVDSAELGKASRIVDAAGRYIEFCKATFPNELSLSELKIVVDCANGATYHIAPNVLRELGANVIAIGCEPNGVNINAEVGATDVRALQARVLAEKADLGIAFDGDGDRVIMVDHEGNKVDGDQIMYIIAREGLRQGQLRGGAVGTLMSNMGLELALKQLGIPFARAKVGDRYVLEKMQEKGWRIGAENSGHVILLDKTTTGDGIVAGLQVLAAMARNHMSLHDLCSGMKMFPQILVNVRYTAGSGDPLEHESVKAVTAEVEAALGNRGRVLLRKSGTEPLIRVMVEGEDEAQVTEFAHRIADAVKAV

SEQ ID NO: 50 - protein, 445 aa, Enterobacteriaceae; identical to SEQ ID NO: 49
  REGION 1..445: note = GlmM, Phosphoglucosamine mutase, GenBank ID: WP_000071134.1

SEQ ID NO: 51 - protein, 456 aa, Escherichia coli K-12
  REGION 1..456: note = GlmU, N-acetylglucosamine-1-phosphate uridyltransferase and glucosamine-1-phosphate acetyltransferase, GenBank ID: NP_418186.1
MLNNAMSVVILAAGKGTRMYSDLPKVLHTLAGKAMVQHVIDAANELGAAHVHLVYGHGGDLLKQALKDDNLNWVLQAEQLGTGHAMQQAAPFFADDEDILMLYGDVPLISVETLQRLRDAKPQGGIGLLTVKLDDPTGYGRITRENGKVTGIVEHKDATDEQRQIQEINTGILIANGADMKRWLAKLTNNNAQGEYYITDIIALAYQEGREIVAVHPQRLSEVEGVNNRLQLSRLERVYQSEQAEKLLLAGVMLRDPARFDLRGTLTHGRDVEIDTNVIIEGNVTLGHRVKIGTGCVIKNSVIGDDCEISPYTVVEDANLAAACTIGPFARLRPGAELLEGAHVGNFVEMKKARLGKGSKAGHLTYLGDAEIGDNVNIGAGTITCNYDGANKFKTIIGDDVFVGSDTQLVAPVTVGKGATIAAGTTVTRNVGENALAISRVPQTQKEGWRRPVKKK

SEQ ID NO: 52 - protein, 456 aa, Enterobacteriaceae; identical to SEQ ID NO: 51
  REGION 1..456: note = GlmU, N-acetylglucosamine-1-phosphate uridyltransferase and glucosamine-1-phosphate acetyltransferase, GenBank ID: WP_000933736.1

SEQ ID NO: 53 - protein, 609 aa, Escherichia coli K-12
  REGION 1..609: note = GlmS, L-glutamine--D-fructose-6-phosphate aminotransferase, GenBank ID: NP_418185.1
MCGIVGAIAQRDVAEILLEGLRRLEYRGYDSAGLAVVDAEGHMTRLRRLGKVQMLAQAAEEHPLHGGTGIAHTRWATHGEPSEVNAHPHVSEHIVVVHNGIIENHEPLREELKARGYTFVSETDTEVIAHLVNWELKQGGTLREAVLRAIPQLRGAYGTVIMDSRHPDTLLAARSGSPLVIGLGMGENFIASDQLALLPVTRRFIFLEEGDIAEITRRSVNIFDKTGAEVKRQDIESNLQYDAGDKGIYRHYMQKEIYEQPNAIKNTLTGRISHGQVDLSELGPNADELLSKVEHIQILACGTSYNSGMVSRYWFESLAGIPCDVEIASEFRYRKSAVRRNSLMITLSQSGETADTLAGLRLSKELGYLGSLAICNVPGSSLVRESDLALMTNAGTEIGVASTKAFTTQLTVLLMLVAKLSRLKGLDASIEHDIVHGLQALPSRIEQMLSQDKRIEALAEDFSDKHHALFLGRGDQYPIALEGALKLKEISYIHAEAYAAGELKHGPLALIDADMPVIVVAPNNELLEKLKSNIEEVRARGGQLYVFADQDAGFVSSDNMHIIEMPHVEEVIAPIFYTVPLQLLAYHVALIKGTDVDQPRNLAKSVTVE

SEQ ID NO: 54 - protein, 609 aa, Enterobacteriaceae; identical to SEQ ID NO: 53
  REGION 1..609: note = GlmS, L-glutamine--D-fructose-6-phosphate aminotransferase, GenBank ID: WP_000334099.1

SEQ ID NO: 55 - protein, 221 aa, Campylobacter jejuni
  REGION 1..221: note = NeuA, CMP-Neu5Ac synthetase, GenBank ID: AAK91728.1
MSLAIIPARGGSKGIKNKNLVLLNNKPLIYYTIKAALNAKSISKVVVSSDSDEILNYAKSQNVDILKRPISLAQDDTTSDKVLLHALKFYKDYEDVVFLQPTSPLRTNIHINEAFNLYKNSNANALISVSECDNKILKAFVCNDCGDLAGICNDEYPFMPRQKLPKTYMSNGAIYILKIKEFLNNPSFLQSKTKHFLMDESSSLDIDCLEDLKKVEQIWKK

SEQ ID NO: 56 - protein, 231 aa, Vibrio brasiliensis
  REGION 1..231: note = NeuA, CMP-Neu5Ac synthetase, GenBank ID: WP_006881452.1
MRVALITARGGSKGLPRKNVLNVNGLPLIGWTINAARECSYIDRVFVSTEDEEIAKISLGMGAELIERPCELAQDNSTSDEVIRHAIDWLDKHSILSDLVVLLQPTSPLRTSAHISEAIDLYDSLNNPNATIISVYEPEHSPLKAFVQLENGTLKGSYNEDAPYTRRQELPKSYLANGAIYIFSPSAFMSESQIPRRDIYPYVMSTNESEDIDSKIDLIRVEKLLRGSFYE

SEQ ID NO: 57 - protein, 346 aa, Campylobacter jejuni
  REGION 1..346: note = NeuB, Neu5 Ac synthase, GenBank ID: AAK91726.1
MKEIKIQNIIISEEKAPLVVPEIGINHNGSLELAKIMVDAAFSAGAKIIKHQTHIVEDEMSKAAKKVIPGNAKISIYEIMQKCALDYKDELALKEYTEKLGLVYLSTPFSRAGANRLEDMGVSAFKIGSGECNNYPLIKHIAAFKKPMIVSTGMNSIESIKPTVKILLDNEIPFVLMHTTNLYPTPHNLVRLNAMLELKKEFSCMVGLSDHTTDNLACLGAVVLGACVLERHFTDSMHRSGPDIVCSMDTKALKELIIQSEQMAIIRGNNESKKAAKQEQVTIDFAFASVVSIKDIKKGEVLSMDNIWVKRPGLGGISAAEFENILGKKALRDIENDAQLSYEDFA

SEQ ID NO: 58 - protein, 346 aa, Flavobacterium limnosediminis
  REGION 1..346: note = NeuB, Neu5 Ac synthase, GenBank ID: WP_023580510.1
MNPYIEIAGRKIGLDYPPLVIAEIGINHEGSLQVAKEIVDAAFRAGVEVVKHQTHIVEDEMSGAAKKVIPGNADVSIYEIMERCALDESEELELKNYVESKGMIFISTPFSRAAAERLKKFDIPAYKIGSGECNNYPLLEHIASFGKPVILSTGMNTVDSIRKAVAIFDKHNVPVALLHTTNLYPTPIHLVRFGAMMEMHNAFPDKVFGLSDHTLNNNACLGAVALGASILERHFTDHMSRTGPDIVCSMDEQATRELIVNSAEIALMRGGTKKPAAEEQVTIDFAFATVCSIAPIKKGEVFTKENIWVKRPGTGKILAEHFERLLGKTATRDIENDEQLDFSDVE

SEQ ID NO: 59 - protein, 372 aa, Campylobacter jejuni
  REGION 1..372: note = NeuC, UDP-GlcNAc 2-epimerase, GenBank AAK91727.1
MKKILFITGSRADYSKIKSLMYRVQNSSEFELYIFATGMHLSKNFGYTVKELYKNGFKNIYEFINYDKYYQTDKALATTIDGFSRYANELKPDLIVVHGDRIEPLAAAIVGALNNILVAHIEGGEISGTIDDSLRHAISKLAHIHLVNDEFAKRRLMQLGEDEKSIFIIGSPDLELLNDNKISLSEAKKYYDINYENYALLMFHPVTTEITSIKNQADNLVKALIQSNKNYIVIYPNNDLGFELILQSYEEFKNNPRFKLFPSLRFEYFITLLKNADFIIGNSSCILKEALYLKTAGILVGSRQNGRLGNENTLKVNANSDEILKAINTIHKKQDLFSAKLEILDSSKLFFEYLQSGDFFKLSTQKVFKDIK

SEQ ID NO: 60 - protein, 391 aa, Enterobacteriaceae
  REGION 1..391: note = NeuC, UDP-GlcNAc 2-epimerase, GenBank ID: WP_000723250.1
MKKILYVTGSRAEYGIVRRLLTMLRETPEIQLDLAVTGMHCDNAYGNTIHIIEQDNFNIIKVVDININTTSHTHILHSMSVCLNSFGDFFSNNTYDAVMVLGDRYEIFSVAIAASMHNIPLIHIHGGEKTLANYDEFIRHSITKMSKLHLTSTEEYKKRVIQLGEKPGSVFNIGSLGAENALSLHLPNKQELELKYGSLLKRYFVVVFHPETLSTQSVNDQIDELLSAISFFKNTHDFIFIGSNADTGSDIIQRKVKYFCKEYKFRYLISIRSEDYLAMIKYSCGLIGNSSSGLIEVPSLKVATINIGDRQKGRVRGASVIDVPVEKNAIVRGINISQDEKFISVVQSSSNPYFKENALINAVRIIKDFIKSKNKDYKDFYDIPECTTSYD

SEQ ID NO: 61 - protein, 391 aa, Escherichia coli S88; identical to SEQ ID NO: 60
  REGION 1..391: note = NeuC, UDP-GlcNAc 2-epimerase, GenBank ID: CAR04561.1

SEQ ID NO: 62 - protein, 392 aa, Pantoea vagans
  REGION 1..392: note = Vag MFS transporter, WP_048785139.1
MKSLLTRKRRINPVFLAFMAASFMIGVAGALQAPTLSLFLTREVQARPLWVGLFFTVNAIAGIVVSMLVAKRSDSRGDRRTLILFCCAMAFCNALLFAFTRHYLTLITLGVLLSALASVSMPQIFALAREYADQSAREAVMFSSVMRAQLSLAWVIGPPLSFALALNFGFVTLFLVAAALFLVCILLIKFTLPSVPRAEPLMRSGGMPLSGWRDRDVRLLFIASVTMWTCNTMYIIDMPLYISVTLGLPEKLAGLLMGTAAGLEIPVMLLAGHYAKRVGKRNLMLIAVAAGVLFYAGLAMFASQTALMALQLFNAVFIGIIAGIGMLWFQDLMPGRPGAATTMFTNSISTGMILAGVIQGTLSERFGHIAVYWLALGLAVAAFAMSARVKNV

SEQ ID NO: 63 - protein, 393 aa, Yersinia frederiksenii
  REGION 1..393: note = Fred MFS transporter, WP_087817556.1
MKSALTFSRRINPVFLAFFVVAFLSGIAGALQAPTLSLFLSTEVKVRPLWVGLFYTVNAIAGITVSFVLAKRSDLRGDRRKLILVCYLMAVGNCLLFAFNRDYLTLITAGVLLAAVANTAMPQIFALAREYADNSAREVVMFSSIMRAQLSLAWVIGPPLSFMLALNYGFTLMFCIAAGIFVLSALVVWFILPSVQRAEPVMDAPTVAQGSLFADKDVLLLFIASMLMWTCNTMYIIDMPLYITASLGLPERLAGLLMGTAAGLEIPIMLLAGYSVRRFGKRKIMLFAVLAGVLFYTGLVLFKFKSALMLLQIFNAIFIGIVAGIGMLYFQDLMPGRAGAATTLFTNSISTGVILAGVLQGVLTETWGHNSVYVMAMILAILSLIICARVREA

SEQ ID NO: 64 - protein, 398 aa, Serratia marcescens
  REGION 1..398: note = Marc MFS transporter, WP_060448169.1
MQRLSRLSLRINPIFAAFLLIAFLSGIAGALLTPTLSLFLTTEVKVRPLWVGLFYTANAVAGIVVSFLLAKRSDTRGDRRRLILLCCLMAVGNCLLFAFNRDYLTLITAGVLMSAVANTAMPQIFALAREYADSEAREVVMFSSVMRAQLSLAWVIGPPLSFALALNYGFTVMFLIAAVTFAVCVLLVGFMLPSVPRAAENEGLQGGVSAPIAPASAWRNRDVRLLFIASMLMWTCNTLYIIDMPLYITADLGLPEGLAGVLMGTAAGLEIPAMLLAGYYVKRFGKRNMMLLAVVAGVLFYLGLTVLESKPALIALQLLNAVFIGIVAGIGMLYFQDLMPGRPGAATTLFTNSISTGVILAGVLQGALVENLGHGSVYWMAALLALAALGMSAKVREV

SEQ ID NO: 65 - protein, 387 aa, Rouxiella badensis
  REGION 1..387: note = Bad MFS transporter, WP_017489914.1
MSSRRLSIIFATFLLVSFLTGIAGALQAPTLSLFLTNEVKVRPLWVGLFYTVNALGGIVISFLLANYSDKKGDRRKLLFFCTLMAIGNSLIFAYSRDYLVLISVGVLLAAIGNASMPQLFALAREYADRSAHEVVMFSSMMRATLSLAWVLGPPISFTLALNYGFTLMYLCAAGVFIFSALMVWFFLPSVGRIEQPVDKVVVHVSAWKNRDVRLLFFASLLMWTCNIMYIIDMPLYITSDLGLPEGLAGLLMGAAAGLEIPVMLIAGYLVKRTGKRRLMLCAAVFGILFYLGLVLFQFKAALMILQLFNAIFIGIIAGIGMLYFQDLMPGRAGSATTLFTNSISTGAILAGVIQGTIVQNFGHYQVYWMALALAVGALVLMTRVKNV

SEQ ID NO: 66 - protein, 394 aa, Rosenbergiella nectarea
  REGION 1..394: note = Nec MFS transporter, WP_092672081.1
MQSFTPPAPKGGNPVFMMFMLVTFFVSIAGALQAPTLSLYLSQELAAKPFMVGLFFTINAVTGIIISFILAKRSDRKGDRRRLLMFCCAMAIANALMFAFVRQYVVLITLGLILSALTSVVMPQLFALAREYADRTGREVVMFSSVMRTQMSLAWVIGPPISFALALNYGFITLYLVAAALFLLSLILIKTTLPSVPRLYPAEDLAKSAASGWKRTDVRFLFAASVLMWVCNLMYIIDMPLYISKSLGMPESFAGVLMGTAAGLEIPVMLLAGYLAKRVGKRPLVIVAAVCGLAFYPAMLVFHQQTGLLIIQLLNAVFIGIVAGLVMLWFQDLMPGKAGAATTLFTNSVSTGMIFAGLCQGLLSDLLGHQAIYVLATVLMVIALLLLLRVKEQA

SEQ ID NO: 67 - protein, 393 aa, Yersinia bercovieri
  REGION 1..393: note = YberC MFS transporter
MKSALTFSRRINPVFLAFFVVAFLSGIAGALQAPTLSLFLSTEVKVRPLWVGLFYTVNAIAGITVSFILAKRSDSRGDRRKLIMVCYLMAVGNCLLFAFNRDYLTLITAGVLLASVANTAMPQIFALAREYADSSAREVVMFSSIMRAQLSLAWVIGPPLSFMLALNYGFTLMFSIAAGIFVLSALVVWFILPSVPRAEPVVDAPVVVQGSLFADKNVLLLFIASMLMWTCNTMYIIDMPLYITASLGLPERLAGLLMGTAAGLEIPIMLLAGYSVRYFGKRKIMLFAVLAGVLFYTGLVLFKFKTALMLLQIFNAIFIGIVAGIGMLYFQDLMPGRAGAATTLFTNSISTGVILAGVLQGGLTETWGHDSVYVMAMVLSILALIICARVREA

SEQ ID NO: 68 - DNA, 107 bp, Escherichia coli
  misc_feature 1..107: note = Plac, lac operon promoter
  source 1..107: mol_type = other DNA
tgtgagttagctcactcattaggcaccccaggctttacactttatgcttccggctcgtatgttgtgtggaattgtgagcggataacaatttcacacaggaaacagct

SEQ ID NO: 69 - DNA, 291 bp, synthetic construct
  misc_feature 1..291: note = PgatY_70UTR, variant of E. coli promoter for gatYZABCD; tagatose-1,6-bisP aldolase
  source 1..291: mol_type = other DNA
cggcaacctatgcctgatgcgacgctgaagcgtcttatcatgcctacatagcactgccacgtatgtttacaccgcatccggcataaaaacacgcgcactttgctacggcttccctatcgggaggccgtttttttgcctttcactcctcgaataattttcatattgtcgtttttgtgatcgttatctcgatatttaaaaacaaataatttcattatattttgtgcctacaagcatcgtggaggtccgtgactttcacgcatacaacaaacattaaccaaggaggaaacagct

SEQ ID NO: 70 - DNA, 300 bp, synthetic construct
  misc_feature 1..300: note = PglpF, E. Coli promoter sequence of glpFKX operon
  source 1..300: mol_type = other DNA
gcggcacgccttgcagattacggtttgccacacttttcatccttctcctggtgacataatccacatcaatcgaaaatgttaataaatttgttgcgcgaatgatctaacaaacatgcatcatgtacaatcagatggaataaatggcgcgataacgctcattttatgacgaggcacacacattttaagttcgatatttctcgtttttgctcgttaacgataagtttacagcatgcctacaagcatcgtggaggtccgtgactttcacgcatacaacaaacattaaccaaggaggaaacagct

SEQ ID NO: 71 - DNA, 300 bp, synthetic construct
  misc_feature 1..300: note = PglpF_SD1, variant of PglpF E. Coli promoter sequence of glpFKX operon
  source 1..300: mol_type = other DNA
gcggcacgccttgcagattacggtttgccacacttttcatccttctcctggtgacataatccacatcaatcgaaaatgttaataaatttgttgcgcgaatgatctaacaaacatgcatcatgtacaatcagatggaataaatggcgcgataacgctcattttatgacgaggcacacacattttaagttcgatatttctcgtttttgctcgttaacgataagtttacagcatgcctacaagcatcgtggaggtccgtgactttcacgcatacaacaaacattaaccaaattcgaaacagct

SEQ ID NO: 72 - DNA, 300 bp, synthetic construct
  misc_feature 1..300: note = PglpF_SD10, variant of PglpF E. Coli promoter sequence of glpFKX operon
  source 1..300: mol_type = other DNA
gcggcacgccttgcagattacggtttgccacacttttcatccttctcctggtgacataatccacatcaatcgaaaatgttaataaatttgttgcgcgaatgatctaacaaacatgcatcatgtacaatcagatggaataaatggcgcgataacgctcattttatgacgaggcacacacattttaagttcgatatttctcgtttttgctcgttaacgataagtttacagcatgcctacaagcatcgtggaggtccgtgactttcacgcatacaacaaacattaaccaactgagaaacagct

SEQ ID NO: 73 - DNA, 300 bp, synthetic construct
  misc_feature 1..300: note = PglpF_SD2, variant of PglpF E. Coli promoter sequence of glpFKX operon
  source 1..300: mol_type = other DNA
gcggcacgccttgcagattacggtttgccacacttttcatccttctcctggtgacataatccacatcaatcgaaaatgttaataaatttgttgcgcgaatgatctaacaaacatgcatcatgtacaatcagatggaataaatggcgcgataacgctcattttatgacgaggcacacacattttaagttcgatatttctcgtttttgctcgttaacgataagtttacagcatgcctacaagcatcgtggaggtccgtgactttcacgcatacaacaaacattaaccaagcgcaaaacagct

SEQ ID NO: 74 - DNA, 300 bp, synthetic construct
  misc_feature 1..300: note = PglpF_SD3 variant of PglpF E. Coli promoter sequence of glpFKX operon
  source 1..300: mol_type = other DNA
gcggcacgccttgcagattacggtttgccacacttttcatccttctcctggtgacataatccacatcaatcgaaaatgttaataaatttgttgcgcgaatgatctaacaaacatgcatcatgtacaatcagatggaataaatggcgcgataacgctcattttatgacgaggcacacacattttaagttcgatatttctcgtttttgctcgttaacgataagtttacagcatgcctacaagcatcgtggaggtccgtgactttcacgcatacaacaaacattaaccaagaacaaaacagct

SEQ ID NO: 75 - DNA, 300 bp, synthetic construct
  misc_feature 1..300: note = PglpF_SD4, variant of PglpF E. Coli promoter sequence of glpFKX operon
  source 1..300: mol_type = other DNA
gcggcacgccttgcagattacggtttgccacacttttcatccttctcctggtgacataatccacatcaatcgaaaatgttaataaatttgttgcgcgaatgatctaacaaacatgcatcatgtacaatcagatggaataaatggcgcgataacgctcattttatgacgaggcacacacattttaagttcgatatttctcgtttttgctcgttaacgataagtttacagcatgcctacaagcatcgtggaggtccgtgactttcacgcatacaacaaacattaaccaactaggaaacagct

SEQ ID NO: 76 - DNA, 300 bp, synthetic construct
  misc_feature 1..300: note = PglpF_SD5, variant of PglpF E. Coli promoter sequence of glpFKX operon
  source 1..300: mol_type = other DNA
gcggcacgccttgcagattacggtttgccacacttttcatccttctcctggtgacataatccacatcaatcgaaaatgttaataaatttgttgcgcgaatgatctaacaaacatgcatcatgtacaatcagatggaataaatggcgcgataacgctcattttatgacgaggcacacacattttaagttcgatatttctcgtttttgctcgttaacgataagtttacagcatgcctacaagcatcgtggaggtccgtgactttcacgcatacaacaaacattaaccaaccgagaaacagct

SEQ ID NO: 77 - DNA, 300 bp, synthetic construct
  misc_feature 1..300: note = PglpF_SD6, variant of PglpF E. Coli promoter sequence of glpFKX operon
  source 1..300: mol_type = other DNA
gcggcacgccttgcagattacggtttgccacacttttcatccttctcctggtgacataatccacatcaatcgaaaatgttaataaatttgttgcgcgaatgatctaacaaacatgcatcatgtacaatcagatggaataaatggcgcgataacgctcattttatgacgaggcacacacattttaagttcgatatttctcgtttttgctcgttaacgataagtttacagcatgcctacaagcatcgtggaggtccgtgactttcacgcatacaacaaacattaaccaagagctaaacagct

SEQ ID NO: 78 - DNA, 300 bp, synthetic construct
  misc_feature 1..300: note = PglpF_SD7, variant of PglpF E. Coli promoter sequence of glpFKX operon
  source 1..300: mol_type = other DNA
gcggcacgccttgcagattacggtttgccacacttttcatccttctcctggtgacataatccacatcaatcgaaaatgttaataaatttgttgcgcgaatgatctaacaaacatgcatcatgtacaatcagatggaataaatggcgcgataacgctcattttatgacgaggcacacacattttaagttcgatatttctcgtttttgctcgttaacgataagtttacagcatgcctacaagcatcgtggaggtccgtgactttcacgcatacaacaaacattaaccaagagcaaaacagct

SEQ ID NO: 79 - DNA, 300 bp, synthetic construct
  misc_feature 1..300: note = PglpF_SD8, variant of PglpF E. Coli promoter sequence of glpFKX operon
  source 1..300: mol_type = other DNA
gcggcacgccttgcagattacggtttgccacacttttcatccttctcctggtgacataatccacatcaatcgaaaatgttaataaatttgttgcgcgaatgatctaacaaacatgcatcatgtacaatcagatggaataaatggcgcgataacgctcattttatgacgaggcacacacattttaagttcgatatttctcgtttttgctcgttaacgataagtttacagcatgcctacaagcatcgtggaggtccgtgactttcacgcatacaacaaacattaaccaagagaaaaacagct

SEQ ID NO: 80 - DNA, 300 bp, synthetic construct
  misc_feature 1..300: note = PglpF_SD9, variant of PglpF E. Coli promoter sequence of glpFKX operon
  source 1..300: mol_type = other DNA
gcggcacgccttgcagattacggtttgccacacttttcatccttctcctggtgacataatccacatcaatcgaaaatgttaataaatttgttgcgcgaatgatctaacaaacatgcatcatgtacaatcagatggaataaatggcgcgataacgctcattttatgacgaggcacacacattttaagttcgatatttctcgtttttgctcgttaacgataagtttacagcatgcctacaagcatcgtggaggtccgtgactttcacgcatacaacaaacattaaccaaaggaaaaacagct

SEQ ID NO: 81 - DNA, 107 bp, synthetic construct
  misc_feature 1..107: note = Plac_16UTR, variant of E. coli lac operon promoter
  source 1..107: mol_type = other DNA
tgtgagttagctcactcattaggcaccccaggctttacactttatgcttccggctcgtatgttgtgtggaattgtgagcggataacaatttcaaggaggaaacagct

SEQ ID NO: 82 - DNA, 203 bp, synthetic construct
  misc_feature 1..203: note = PmglB_70UTR, variant of E. coli promoter for mglBAC galactose/methyl-galactosidade transporter
  source 1..203: mol_type = other DNA
tgcgtcgccattctgtcgcaacacgccagaatgcggcggcgatcactaactcaacaaatcaggcgatgtaaccgctttcaatctgtgagtgatttcacagtatcttaacaatgtgatagctatgattgcaccgtgcctacaagcatcgtggaggtccgtgactttcacgcatacaacaaacattaaccaaggaggaaacagct

SEQ ID NO: 83 - DNA, 203 bp, synthetic construct
  misc_feature 1..203: note = PmglB_70UTR_SD4, variant of E. coli promoter for mglBAC; galactose/methyl-galactosidade transporter
  source 1..203: mol_type = other DNA
tgcgtcgccattctgtcgcaacacgccagaatgcggcggcgatcactaactcaacaaatcaggcgatgtaaccgctttcaatctgtgagtgatttcacagtatcttaacaatgtgatagctatgattgcaccgtgcctacaagcatcgtggaggtccgtgactttcacgcatacaacaaacattaaccaactaggaaacagct

SEQ ID NO: 84 - DNA, 76 bp, synthetic construct
  misc_feature 1..76: note = CP6 promotor sequence
  source 1..76: mol_type = other DNA
catgtgggagtttattcttgacacagatatttccggatgatataataactgagtactgttcacacaggaaacagct

SEQ ID NO: 85 - DNA, 269 bp, Escherichia coli
  misc_feature 1..269: note = PosmY, promotor for osmY-ytjA; perplasmic chaperone
  source 1..269: mol_type = other DNA
caaaattgtgatctatatttaacaaagtgatgacatttctgacggcgttaaataccgttcaatgcgtagatatcagtatctaaagccgtcgattgtcattctaccgatattaataactgattcagaggctgtaatggtcgttattcatcactcatcgcttttgtgatggcgaccattgacttctgtagagggtgaagtctctccctattcagcaatgcaacctcgtgttgccaggctcaaattacgagcaaaccaaggaggaaacagct

SEQ ID NO: 86 - protein, 483 aa, Avibacterium gallinarum
  REGION 1..483: note = SacC_Agal, glycoside hydrolase family 32 protein, WP_103853210.1
MIIFNEGKYKSLYAAEQGELEKIAQTVAQDQDFRPVYHLAPPTGLLNDPNGLIFDGEKYHLFYQWYPFDALHGMKHWQHFITQDFKQFSQADLLVPCELYESHGCYSGGAVKIGDQIAVFYTGNTRRPSDNQRVPYQNLAIFSKDGKLLSKRPLIEQAPQGYTEHVRDPKPFLTKDGKIRFICGAQRENLTGTALVFEMDNLADTPRLLGELALPAFDNQGVFMWECPDLSQMGDKSLFIWSPQGKARELEQYQNNYHAVYALGELADRQFHAEQIAELDQGFDFYAPQTFSGTQTMLLGWVGLPDLSYPTDLYKWHSMLSMPRQLRLQDGKIYQQPIENIYKNLTALQSITVEKEAEIADLDRAYLKFDANAQPFSLKFFNNAQNQRLILSYDGEMLCLDRSQTEQTDSMKSFGDKRYCRIEDLRQVEIFFDRSVAEIFLNQGEKAMTSRFFICARENQLCTDKPLTLQVGYPKKIEVDYTK

SEQ ID NO: 87 - protein, 548 aa, Arthrobacter globiformis
  REGION 1..548: note = Bff, beta-fructofuranosidase protein, BAD18121.1
MERTCITVRAIVRFHIEQRQTIVNKQRTKRGILTAALSIGALGATLISGPAVAATDAAPGFPQPTEHTQKAYSPTDNFTSRWTRADAKQLKAMSDPDAGSRENSMPTEYTMPTVSQDFPDMSNEKVWVWDTWPLIDENANQYSVNGQEIIFSLVADRKLGFDERHQYARIGYFYRPAGIPADERPEDGGWTYGGQVFDEGVTGKIFEDQSFTHQTQWSGSARVSKNGEIKLFFTDVAFYRDKDGQDVKPYDSRIALSVGHVHSNKKGVKLTGFNKVKELLQADGKNYQNAAQNSYYNFRDPFTFVDPAHPGETYMVFEGNSAMDRDEAKCTAEDLGYREGETNGETVEQVNNSGATYQIGNVGLARAKNKALTEWEFLPPILSANCVTDQTERPQIYMQDGKYYLFTISHRSTFATGIDGPEGVYGFVGNGIRSDYQPLNRGSGLALGSPTNLNFAAGTPFAPDYNQHPGQFQAYSHYVMPGGLVQSFIDTIGTKDNFVRGGTLGPTVKLNIKGDSATVDYNYGDNGLGGWADIPANRELKNSKAVAK

SEQ ID NO: 88 - protein, 505 aa, Klebsiella pneumoniae
  REGION 1..505: note = ScrY, sucrose porin, GeneBank ID CAA40657.1
MYKKRKLAILIALLTGTAAAHGQTDLNSIEARLAALEKRLQDAETRASTAESRAASAEQKVQQLTQQQQQTQATTQQVARRTTQLEEKAERPGGFEFHGYARSGVIMNDSAASTKSGAYMTPAGETGGAIGRLGNQADTYVEMNLEHKQTLDNGATTRFKVMVADGQTTYNDWTASSSDLNVRQAFVELGNLPTFEGPFKGSTLWAGKRFDRDNFDIHWIDSDVVFLAGTGGGIYDVKWNDSLRSNFSLYGRNFGDIADSSNSVQNYIVSMNNFAGPVQMMVSGMRAKDNDDRQDANGNLVKGDAANTGVHALLGLHNESFYGLRDGTSKTALLYGHGLGAEVKGIGSDGALRPGANTWRFASYGTTPLSDRWFIAPAVLAQSSKDRYVDGDSYQWATLNLRLIQEVTQNFALAWEGSYQYMDLQPEGYNDRHAVNGSFYKLTFAPTFKVGSIGDFFSRPEIRFYTSWMDWSKKLDNYANDDALGSNGFKSGGEWSFGMQMETWF

SEQ ID NO: 89 - protein, 456 aa, Klebsiella pneumoniae
  REGION 1..456: note = ScrA, sucrose-specific enzyme II, GeneBank ID: CAA40658.1
MDFEQISRSLLPLLGGKENIASAAHCATRLRLVLVDDALADQQAIGKIDGVKGCFRNAGQMQIIFGTGVVNKVYAAFIQAAGISESSKSEAADLAAKKLNPFQRIARLLSNIFVPIIPAIVASGLLMGLLGMVKTYGWVDPSNALYIMLDMCSSAAFIILPILIGFTAAREFGGNPYLGATLGGILTHPALTNAWGVAAGFHTMNFFGIEVAMIGYQGTVFPVLLAVWFMSMVEKRLRRVIPDALDLILTPFLTVIISGFIALLLIGPAGRALGDGISFILSTLISHAGWLAGLLFGGLYSVIVITGIHHSFHAIEAGLLGNPSIGVNFLLPIWAMANVAQGGACFAVWFKTKDAKIKAITLPSAFSAMLGITEAAIFGINLRFVKPFIAALVGGAAGGAWVVSMHVYMTAVGLTAIPGMAIVQASSLLNYIIGMAIAFAVAFALSLTLKYKTDAE

SEQ ID NO: 90 - protein, 466 aa, Salmonella enterica subsp. enterica serovar Typhimurium
  REGION 1..466: note = ScrB, beta-fructofuranosidase, GeneBank ID: CAA47974.1
MSLPSRLPAILQAVMQGQPRALADSHYPRWHHAPVTGLMNDPNGFIEFAGRYHLFYQWNPLACDHTFKCWAHWSSIDLLHWQHEPIALMPDEEYDRNGCYSGSAVDNNGTLTLCYTGNVKFAEGGRTAWQCLATENADGTFRKIGPVLPLPEGYTGHVRDPKVWRHEDLWYMVLGAQDRQKRGKVLLFSSADLHQWTSMGEIAGHGINGLDDVGYMWECPDLFPLGDQHILICCPQGIAREEECYLNTYPAVWMAGEFDYAAGAFRHGELHELDAGFEFYAPQTMLTSDGRRLLVGWMGVPEGEEMLQPTLNNGWIHQMTCLRELEFINGQLYQRPLRELSALRGEANGWSGNALPLAPMEIDLQTRGGDMLSLDFGGVLTLECDASGLRLARRSLASDEMHYRYWRGNVRSLRVFIDQSSVEIFINGGEGVMSSRYFPACSGQLTFSGITPDAFCYWPLRTCMVE

SEQ ID NO: 91 - protein, 334 aa, Salmonella enterica subsp. enterica serovar Typhimurium
  REGION 1..334: note = ScrR, sucrose repressor, GeneBank ID: CAA47975.1
MKTKRVTIKDIAEQAGVSKATASLVLNGRGKELRVAQETRERVLSIARKHHYQPSIHARSLRNNRSHTIGLVVPEITNHGFAVFAHELEMLCREAGVQLLISCTDENPGQESVVVNNMIARQVDGMIVASCMHNDADYLKLSQQLPVVLFDRCPNESALPLVMTDSITPTAELISRIAPQHSDEFWFLGGQARLSPSRDRLTGFTQGLAQAGIALRPEWVINGNYHPSSGYEMFAALCARLGRPPKALFTAACGLLEGVLRYMSQHHLLDSDIHLTSFDDHYLYDSLSLRIDTVQQDNRQLAWHCYDLISQLIEGDTPETLQRYLPATLQFRHQ

SEQ ID NO: 92 - DNA, 730 bp, Escherichia coli
  misc_feature 1..730: note = glpR coding sequence
  source 1..730: mol_type = genomic DNA
atgaaacaaacacaacgtcacaacggtattatcgaactggttaaacagcagggttatgtcagtaccgaagagctggtagagcatttctccgtcagcccgcagactattcgccgcgacctcaatgagctggcggagcaaaacctgatcctggccatcatggcggtgcggcgctgccttccagttcggttaacacgccgtggcacgatcgcaaggccacccagaccgaagaaaaagagcgcatcgcccgcaaagtggcggagcaaatccccaatggctcgacgctgtttatcgatatcggcaccacgccggaagcggtagcgcacgcactgctcaatcacagcaatttgcgcattgtcaccaacaatctcaacgttgctaacacgttgatggtaaaagaagattttcgcatcattctcgccggtggcgaattacgcagccgcgatggcgggatcattggcgaagcgacgctcgattttatctcccagttccgccttgatttcggcattctggggataagcggcatcgatagcgacggctcgctgctggagttcgattaccacgaagttcgcaccaaacgcgccattattgagaactcgcgccacgttatgctggttgtcgatcactcgaaatttggccgtaacgcgatggtcaatatgggcagcatcagcatggtagatgccgtctacaccgacgccccgccgccagtaagcgtgatgcaggtgctgacgga

SEQ ID NO: 93 - DNA, 203 bp, synthetic construct
  misc_feature 1..203: note = PmglB_70UTR_SD8 promoter sequence
  source 1..203: mol_type = other DNA
tgcgtcgccattctgtcgcaacacgccagaatgcggcggcgatcactaactcaacaaatcaggcgatgtaaccgctttcaatctgtgagtgatttcacagtatcttaacaatgtgatagctatgattgcaccgtgcctacaagcatcgtggaggtccgtgactttcacgcatacaacaaacattaaccaagagaaaaacagct

SEQ ID NO: 94 - DNA, 203 bp, synthetic construct
  misc_feature 1..203: note = PmglB_70UTR_SD10 promoter sequence
  source 1..203: mol_type = other DNA
tgcgtcgccattctgtcgcaacacgccagaatgcggcggcgatcactaactcaacaaatcaggcgatgtaaccgctttcaatctgtgagtgatttcacagtatcttaacaatgtgatagctatgattgcaccgtgcctacaagcatcgtggaggtccgtgactttcacgcatacaacaaacattaaccaactgagaaacagct

SEQ ID NO: 95 - DNA, 203 bp, synthetic construct
  misc_feature 1..203: note = PmglB-54UTR promoter sequence
  source 1..203: mol_type = other DNA
tgcgtcgccattctgtcgcaacacgccagaatgcggcggcgatcactaactcaacaaatcaggcgatgtaaccgctttcaatctgtgagtgatttcacagtatcttaacaatgtgatagctatgattgcaccgtgcctacaagcatcgtggaggtccgtgactttcacgcatacaacaaacattaacaaaaaccggagatacc

SEQ ID NO: 96 - DNA, 141 bp, synthetic construct
  misc_feature 1..141: note = Plac 70_UTR promoter sequence
  source 1..141: mol_type = other DNA
tgtgagttagctcactcattaggcaccccaggctttacactttatgcttccggctcgtatgttgtgtggaatgcctacaagcatcgtggaggtccgtgactttcacgcatacaacaaacattaaccaaggaggaaacagct

SEQ ID NO: 97 - DNA, 203 bp, synthetic construct
  misc_feature 1..203: note = PmglB_70UTR_SD9 promoter sequence
  source 1..203: mol_type = other DNA
tgcgtcgccattctgtcgcaacacgccagaatgcggcggcgatcactaactcaacaaatcaggcgatgtaaccgctttcaatctgtgagtgatttcacagtatcttaacaatgtgatagctatgattgcaccgtgcctacaagcatcgtggaggtccgtgactttcacgcatacaacaaacattaaccaaaggaaaaacagct

SEQ ID NO: 98 - DNA, 203 bp, synthetic construct
  misc_feature 1..203: note = PmglB_70UTR_SD5 promoter sequence
  source 1..203: mol_type = other DNA
tgcgtcgccattctgtcgcaacacgccagaatgcggcggcgatcactaactcaacaaatcaggcgatgtaaccgctttcaatctgtgagtgatttcacagtatcttaacaatgtgatagctatgattgcaccgtgcctacaagcatcgtggaggtccgtgactttcacgcatacaacaaacattaaccaaccgagaaacagct

SEQ ID NO: 99 - DNA, 203 bp, synthetic construct
  misc_feature 1..203: note = PmglB_70UTR_SD7 promoter sequence
  source 1..203: mol_type = other DNA
tgcgtcgccattctgtcgcaacacgccagaatgcggcggcgatcactaactcaacaaatcaggcgatgtaaccgctttcaatctgtgagtgatttcacagtatcttaacaatgtgatagctatgattgcaccgtgcctacaagcatcgtggaggtccgtgactttcacgcatacaacaaacattaaccaagagcaaaacagct

SEQ ID NO: 100 - DNA, 189 bp, synthetic construct
  misc_feature 1..189: note = PglpA_70UTR promoter sequence
  source 1..189: mol_type = other DNA
gaaaacattcataaattaaatgtgaattgccgcacacattattaaataagatttacaaaatgttcaaaatgacgcatgaaatcacgtttcactttcgaattatgagcgaatatgcgcgatgcctacaagcatcgtggaggtccgtgactttcacgcatacaacaaacattaaccaaggaggaaacagct

SEQ ID NO: 101 - DNA, 239 bp, synthetic construct
  misc_feature 1..239: note = PglpT_70UTR promoter sequence
  source 1..239: mol_type = other DNA
ccatttagccatagtaaaaacatgaattgtttgatttcgcgcatattcgctcataattcgaaagtgaaacgtgatttcatgcgtcattttgaacattttgtaaatcttatttaataatgtgtgcggcaattcacatttaatttatgaatgttttcttaacatcgcggcatgcctacaagcatcgtggaggtccgtgactttcacgcatacaacaaacattaaccaaggaggaaacagct

SEQ ID NO: 102 - DNA, 350 bp, synthetic construct
  misc_feature 1..350: note = PmglB_16UTR promoter sequence
  source 1..350: mol_type = other DNA
tgcgtcgccattctgtcgcaacacgccagaatgcggcggcgatcactaactcaacaaatcaggcgatgtaaccgctttcaatctgtgagtgatttcacagtatcttaacaatgtgatagctatgattgcaccgttttaacgttgtaacccgtatgtaacagtgaataatcacttttgccgaggtaacagcgtcataacaacaattaaagccgttttctggagcgttaccgggcatggaagaacgaattttaaaaagtgagcttcggcgttcagtaacacttcattaactctactgccccgccgagcatttatctcaagcactaccctgcataagcaaggaggaaacagct

SEQ ID NO: 103 - DNA, 189 bp, synthetic construct; identical to SEQ ID NO: 100
  misc_feature 1..189: note = PglpA_16UTR promoter sequence
  source 1..189: mol_type = other DNA